European Patent Application EP 4 491 615 A1, published January 15, 2025. Title: LIPIDS AND USES THEREOF. Applicant: TAIWAN BIO-MANUFACTURING CORPORATION. Application EP. The sequence listing filed with the application follows.

SEQUENCE LISTING (1 sequence)

SEQ ID NO: 1 - RNA, 1653 nt, synthetic construct
  source 1..1653: mol_type = other RNA
atggaggacgccaagaacatcaagaagggccccgcccccttctaccccctggaggacggcaccgccggcgagcagctgcacaaggccatgaagcggtacgccctggtgcccggcaccatcgccttcaccgacgcccacatcgaggtggacatcacctacgccgagtacttcgagatgagcgtgcggctggccgaggccatgaagcggtacggcctgaacaccaaccaccggatcgtggtgtgcagcgagaacagcctgcagttcttcatgcccgtgctgggcgccctgttcatcggcgtggccgtggcccccgccaacgacatctacaacgagcgggagctgctgaacagcatgggcatcagccagcccaccgtggtgttcgtgagcaagaagggcctgcagaagatcctgaacgtgcagaagaagctgcccatcatccagaagatcatcatcatggacagcaagaccgactaccagggcttccagagcatgtacaccttcgtgaccagccacctgccccccggcttcaacgagtacgacttcgtgcccgagagcttcgaccgggacaagaccatcgccctgatcatgaacagcagcggcagcaccggcctgcccaagggcgtggccctgccccaccggaccgcctgcgtgcggttcagccacgcccgggaccccatcttcggcaaccagatcatccccgacaccgccatcctgagcgtggtgcccttccaccacggcttcggcatgttcaccaccctgggctacctgatctgcggcttccgggtggtgctgatgtaccggttcgaggaggagctgttcctgcggagcctgcaggactacaagatccagagcgccctgctggtgcccaccctgttcagcttcttcgccaagagcaccctgatcgacaagtacgacctgagcaacctgcacgagatcgccagcggcggcgcccccctgagcaaggaggtgggcgaggccgtggccaagcggttccacctgcccggcatccggcagggctacggcctgaccgagaccaccagcgccatcctgatcacccccgagggcgacgacaagcccggcgccgtgggcaaggtggtgcccttcttcgaggccaaggtggtggacctggacaccggcaagaccctgggcgtgaaccagcggggcgagctgtgcgtgcggggccccatgatcatgagcggctacgtgaacaaccccgaggccaccaacgccctgatcgacaaggacggctggctgcacagcggcgacatcgcctactgggacgaggacgagcacttcttcatcgtggaccggctgaagagcctgatcaagtacaagggctaccaggtggcccccgccgagctggagagcatcctgctgcagcaccccaacatcttcgacgccggcgtggccggcctgcccgacgacgacgccggcgagctgcccgccgccgtggtggtgctggagcacggcaagaccatgaccgagaaggagatcgtggactacgtggccagccaggtgaccaccgccaagaagctgcggggcggcgtggtgttcgtggacgaggtgcccaagggcctgaccggcaagctggacgcccggaagatccgggagatcctgatcaaggccaagaagggcggcaagatcgccgtgtga